European Patent Application EP 4 183 393 A1, published May 24, 2023. Title: Compounds for the treatment of hepatocellular carcinoma. Applicant: Servicio Andaluz de Salud Universidad de Córdoba. The sequence listing filed with the application follows.

SEQUENCE LISTING (2 sequences)

SEQ ID NO: 1 - protein, 1304 aa, Homo sapiens
MAKIAKTHEDIEAQIREIQGKKAALDEAQGVGLDSTGYYDQEIYGGSDSRFAGYVTSIAATELEDDDDDYSSSTSLLGQKKPGYHAPVALLNDIPQSTEQYDPFAEHRPPKIADREDEYKKHRRTMIISPERLDPFADGGKTPDPKMNARTYMDVMREQHLTKEEREIRQQLAEKAKAGELKVVNGAAASQPPSKRKRRWDQTADQTPGATPKKLSSWDQAETPGHTPSLRWDETPGRAKGSETPGATPGSKIWDPTPSHTPAGAATPGRGDTPGHATPGHGGATSSARKNRWDETPKTERDTPGHGSGWAETPRTDRGGDSIGETPTPGASKRKSRWDETPASQMGGSTPVLTPGKTPIGTPAMNMATPTPGHIMSMTPEQLQAWRWEREIDERNRPLSDEELDAMFPEGYKVLPPPAGYVPIRTPARKLTATPTPLGGMTGFHMQTEDRTMKSVNDQPSGNLPFLKPDDIQYFDKLLVDVDESTLSPEEQKERKIMKLLLKIKNGTPPMRKAALRQITDKAREFGAGPLFNQILPLLMSPTLEDQERHLLVKVIDRILYKLDDLVRPYVHKILVVIEPLLIDEDYYARVEGREIISNLAKAAGLATMISTMRPDIDNMDEYVRNTTARAFAVVASALGIPSLLPFLKAVCKSKKSWQARHTGIKIVQQIAILMGCAILPHLRSLVEIIEHGLVDEQQKVRTISALAIAALAEAATPYGIESFDSVLKPLWKGIRQHRGKGLAAFLKAIGYLIPLMDAEYANYYTREVMLILIREFQSPDEEMKKIVLKVVKQCCGTDGVEANYIKTEILPPFFKHFWQHRMALDRRNYRQLVDTTVELANKVGAAEIISRIVDDLKDEAEQYRKMVMETIEKIMGNLGAADIDHKLEEQLIDGILYAFQEQTTEDSVMLNGFGTVVNALGKRVKPYLPQICGTVLWRLNNKSAKVRQQAADLISRTAVVMKTCQEEKLMGHLGVVLYEYLGEEYPEVLGSILGALKAIVNVIGMHKMTPPIKDLLPRLTPILKNRHEKVQENCIDLVGRIADRGAEYVSAREWMRICFELLELLKAHKKAIRRATVNTFGYIAKAIGPHDVLATLLNNLKVQERQNRVCTTVAIAIVAETCSPFTVLPALMNEYRVPELNVQNGVLKSLSFLFEYIGEMGKDYIYAVTPLLEDALMDRDLVHRQTASAVVQHMSLGVYGFGCEDSLNHLLNYVWPNVFETSPHVIQAVMGALEGLRVAIGPCRMLQYCLQGLFHPARKVRDVYWKIYNSIYIGSQDALIAHYPRIYNDDKNTYIRYELDYIL

SEQ ID NO: 2 - DNA, 6463 bp, Homo sapiens
agttccgtctgtgtgttcgagtggacaaaatggcgaagatcgccaagactcacgaagatattgaagcacagattcgagaaattcaaggcaagaaggcagctcttgatgaagctcaaggagtgggcctcgattctacaggttattatgaccaggaaatttatggtggaagtgacagcagatttgctggatacgtgacatcaattgctgcaactgaacttgaagatgatgacgatgactattcatcatctacgagtttgcttggtcagaagaagccaggatatcatgcccctgtggcattgcttaatgatataccacagtcaacagaacagtatgatccatttgctgagcacagacctccaaagattgcagaccgggaagatgaatacaaaaagcataggcggaccatgataatttccccagagcgtcttgatccttttgcagatggagggaaaacccctgatcctaaaatgaatgctaggacttacatggatgtaatgcgagaacaacacttgactaaagaagaacgagaaattaggcaacagctagcagaaaaagctaaagctggagaactaaaagtcgtcaatggagcagcagcgtcccagcctccatcaaaacgaaaacggcgttgggatcaaacagctgatcagactcctggtgccactcccaaaaaactatcaagttgggatcaggcagagacccctgggcatactccttccttaagatgggatgagacaccaggtcgtgcaaagggaagcgagactcctggagcaaccccaggctcaaaaatatgggatcctacacctagccacacaccagcgggagctgctactcctggacgaggtgatacaccaggccatgcgacaccaggccatggaggcgcaacttccagtgctcgtaaaaacagatgggatgaaacccccaaaacagagagagatactcctgggcatggaagtggatgggctgagactcctcgaacagatcgaggtggagattctattggtgaaacaccgactcctggagccagtaaaagaaaatcacggtgggatgaaacaccagctagtcagatgggtggaagcactccagttctgacccctggaaagacaccaattggcacaccagccatgaacatggctacccctactccaggtcacataatgagtatgactcctgaacagcttcaggcttggcggtgggaaagagaaattgatgagagaaatcgcccactttctgatgaggaattagatgctatgttcccagaaggatataaggtacttcctcctccagctggttatgttcctattcgaactccagctcgaaagctgacagctactccaacacctttgggtggtatgactggtttccacatgcaaactgaagatcgaactatgaaaagtgttaatgaccagccatctggaaatcttccatttttaaaacctgatgatattcaatactttgataaactattggttgatgttgatgaatcaacacttagtccagaagagcaaaaagagagaaaaataatgaagttgcttttaaaaattaagaatggaacaccaccaatgagaaaggctgcattgcgtcagattactgataaagctcgtgaatttggagctggtcctttgtttaatcagattcttcctctgctgatgtctcctacacttgaggatcaagagcgtcatttacttgtgaaagttattgataggatactgtacaaacttgatgacttagttcgtccatatgtgcataagatcctcgtggtcattgaaccgctattgattgatgaagattactatgctagagtggaaggccgagagatcatttctaatttggcaaaggctgctggtctggctactatgatctctaccatgagacctgatatagataacatggatgagtatgtccgtaacacaacagctagagcttttgctgttgtagcctctgccctgggcattccttctttattgcccttcttaaaagctgtgtgcaaaagcaagaagtcctggcaagcgagacacactggtattaagattgtacaacagatagctattcttatgggctgtgccatcttgccacatcttagaagtttagttgaaatcattgaacatggtcttgtggatgagcagcagaaagttcggaccatcagtgctttggccattgctgccttggctgaagcagcaactccttatggtatcgaatcttttgattctgtgttaaagcctttatggaagggtatccgccaacacagaggaaagggtttggctgctttcttgaaggctattgggtatcttattcctcttatggatgcagaatatgccaactactatactagagaagtgatgttaatccttattcgagaattccagtctcctgatgaggaaatgaaaaaaattgtgctgaaggtggtaaaacagtgttgtgggacagatggtgtagaagcaaactacattaaaacagagattcttcctcccttttttaaacacttctggcagcacaggatggctttggatagaagaaattaccgacagttagttgatactactgtggagttggcaaacaaagtaggtgcagcagaaattatatccaggattgtggatgatctgaaagatgaagccgaacagtacagaaaaatggtgatggagacaattgagaaaattatgggtaatttgggagcagcagatattgatcataaacttgaagaacaactgattgatggtattctttatgctttccaagaacagactacagaggactcagtaatgttgaacggctttggcacagtggttaatgctcttggcaaacgagtcaaaccatacttgcctcagatctgtggtacagttttgtggcgtttaaataacaaatctgctaaagttaggcaacaggcagctgacttgatttctcgaactgctgttgtcatgaagacttgtcaagaggaaaaattgatgggacacttgggtgttgtattgtatgagtatttgggtgaagagtaccctgaagtattgggcagcattcttggagcactgaaggccattgtaaatgtcataggtatgcataagatgactccaccaattaaagatctgctgcctagactcacccccatcttaaagaacagacatgaaaaagtacaagagaattgtattgatcttgttggtcgtattgctgacaggggagctgaatatgtatctgcaagagagtggatgaggatttgctttgagcttttagagctcttaaaagcccacaaaaaggctattcgtagagccacagtcaacacatttggttatattgcaaaggccattggccctcatgatgtattggctacacttctgaacaacctcaaagttcaagaaaggcagaacagagtttgtaccactgtagcaatagctattgttgcagaaacatgttcaccctttacagtactccctgccttaatgaatgaatacagagttcctgaactgaatgttcaaaatggagtgttaaaatcgctttccttcttgtttgaatatattggtgaaatgggaaaagactacatttatgccgtaacaccgttacttgaagatgctttaatggatagagaccttgtacacagacagacggctagtgcagtggtacagcacatgtcacttggggtttatggatttggttgtgaagattcgctgaatcacttgttgaactatgtatggcccaatgtatttgagacatctcctcatgtaattcaggcagttatgggagccctagagggcctgagagttgctattggaccatgtagaatgttgcaatattgtttacagggtctgtttcacccagcccggaaagtcagagatgtatattggaaaatttacaactccatctacattggttcccaggacgctctcatagcacattacccaagaatctacaacgatgataagaacacctatattcgttatgaacttgactatatcttataattttattgtttattttgtgtttaatgcacagctacttcacaccttaaacttgctttgatttggtgatgtaaacttttaaacattgcagatcagtgtagaactggtcatagaggaagagctagaaatccagtagcatgatttttaaataacctgtctttgtttttgatgttaaacagtaaatgccagtagtgaccaagaacacagtgattatatacactatactggagggatttcatttttaattcatctttatgaagatttagaactcattccttgtgtttaaagggaatgtttaattgagaaataaacatttgtgtacaaaatgctaatttgtgtgtgttttttgaacatgacttgtaaaatgcggaactttgataaagtattggtttatgtggaataagtggcttaatttcattttctgtcacatggtttatagaaagtagttagctgaataaaaactatataaagtgatggcatctttgtcaaaattccattgttgtgttaataatgacagcaagaagagtagcctcaggggatgttcccctcaaactagcacaaccattccatcatcgtagaaaagtagcacttttgctaaactgtcttgaatattttgtacttacatagcgcctttcatctcttgatttctcaaaatgctttatgaacacatttaaagaaagtggtttaagtcttgtccaacacttgacaggtctgctgtgtttagcaagtgaggaatttaactttacttcaaaactgctttctgcctattaggagtgaggatacctaagtaatgctgatagaacaggacaatgttgggcttttctccatgttataagccactactcagcaatgcatcagtaaatacctattcacccactgtatgccagccactgtgcttatatgcaggggatgcaaaggtgcatgagacctgccctctacctttaagaacagtataatggagaaggggagacaaaccttgtgacagattccttatgtactgtgataatacacagtggcagcagctaaaatgtctaggtttgcttagctttgtattcagtaataataagttgatctaagagttcagcataaactgaatgaaatgccatttaatggtagaggaaccaagcattaaggcagtactacacttaattttttaagcaaatatgtaaagtatattttcaaacttttctaatgttatggccccaaatttcttagttttggcctttttactacctatactatttttactgttttgttttgtctccatgtggtagtacttctgtgaactctaaagggaaaaaaaattctgcaagcagcattagtatataactactactgtaagtaaaactgcctattgacactttaggagttcctgcttcagaagcttagttaagaaacagcttgtggccgggtgtggtggctcatgcctgtaatcccagcactttgggaggctgaggcgggcggatcacgaggtcaggagatcgagaccatcctggctaacgcggtgaagtcccgtctactaaaaatacaaaaattagccaggcgtggtggcgggcgcctgtagtcccagctactagggaggctgaggcaggagaatggcttgaacccgggaggcggagcttgcagtgagccgagatagcgctgctacactccagcctgggcgacagagactccgtctcaaaaaaaaaaaaaaaattgactttcaacaaattgatagtgagcattaagggtttccaagttggatttgtaactcctcatcattccttgtatgacaactttctgaatatatgtcactatgtagtaaaattaaacactccaaactcatctttctgttgttagaagttttcagcggtacttccatgcaactttaaatctcactgctctctatggttgatgtcaaatgaccttcagtaatgactgagaattgaatacaaatagattacaaagccaaaatttgatgttaaatgactcaggaaattttagttgtattttcaattcaagtacttagtagcctacgtttgcttggcctctggttctttatggaaaataggctttgtagtggcattgtggagcaaaggagactgttacaccttaattaactttttttactgatgcaaataatttgaggatagagaggagggaagtagtgaaagctatgacctaaaacattgggaccaaatagaggctcacagatatttggattattttatgtgcttattattaaataaggaaagcattttgtgatatgtggaagacgctatgtgaagttttacctatcttctcaaagaccttttcttttgtattttcttttggtgtttcttaaagccaaacaaagaaatgttcttaaggagacagggtgggtttttctgtgggcctttgttggtttttctgtgggccatcgccctctaatggaattgatctctggctgtttgatttttttcatattgtatttttaaaatttgttgtacagtgccctgtgagcaccaagtaccactagatgaataaaacgtattatatctaaa